European Patent Specification EP 3 808 770 B1, published October 29, 2025. Title: ANTI-HUMAN THYROGLOBULIN T CELL RECEPTORS. Applicant: THE UNITED STATES OF AMERICA, AS REPRESENTED BY THE SECRETARY, DEPARTMENT OF HEALTH AND HUMAN SERVICES. The sequence listing filed with the application follows.

SEQUENCE LISTING (58 sequences)

SEQ ID NO: 1 - protein, 2768 aa, Homo sapiens
MALVLEIFTLLASICWVSANIFEYQVDAQPLRPCELQRETAFLKQADYVPQCAEDGSFQTVQCQNDGRSCWCVGANGSEVLGSRQPGRPVACLSFCQLQKQQILLSGYINSTDTSYLPQCQDSGDYAPVQCDVQQVQCWCVDAEGMEVYGTRQLGRPKRCPRSCEIRNRRLLHGVGDKSPPQCSAEGEFMPVQCKFVNTTDMMIFDLVHSYNRFPDAFVTFSSFQRRFPEVSGYCHCADSQGRELAETGLELLLDEIYDTIFAGLDLPSTFTETTLYRILQRRFLAVQSVISGRFRCPTKCEVERFTATSFGHPYVPSCRRNGDYQAVQCQTEGPCWCVDAQGKEMHGTRQQGEPPSCAEGQSCASERQQALSRLYFGTSGYFSQHDLFSSPEKRWASPRVARFATSCPPTIKELFVDSGLLRPMVEGQSQQFSVSENLLKEAIRAIFPSRGLARLALQFTTNPKRLQQNLFGGKFLVNVGQFNLSGALGTRGTFNFSQFFQQLGLASFLNGGRQEDLAKPLSVGLDSNSSTGTPEAAKKDGTMNKPTVGSFGFEINLQENQNALKFLASLLELPEFLLFLQHAISVPEDVARDLGDVMETVLSSQTCEQTPERLFVPSCTTEGSYEDVQCFSGECWCVNSWGKELPGSRVRGGQPRCPTDCEKQRARMQSLMGSQPAGSTLFVPACTSEGHFLPVQCFNSECYCVDAEGQAIPGTRSAIGKPKKCPTPCQLQSEQAFLRTVQALLSNSSMLPTLSDTYIPQCSTDGQWRQVQCNGPPEQVFELYQRWEAQNKGQDLTPAKLLVKIMSYREAASGNFSLFIQSLYEAGQQDVFPVLSQYPSLQDVPLAALEGKRPQPRENILLEPYLFWQILNGQLSQYPGSYSDFSTPLAHFDLRNCWCVDEAGQELEGMRSEPSKLPTCPGSCEEAKLRVLQFIRETEEIVSASNSSRFPLGESFLVAKGIRLRNEDLGLPPLFPPREAFAEQFLRGSDYAIRLAAQSTLSFYQRRRFSPDDSAGASALLRSGPYMPQCDAFGSWEPVQCHAGTGHCWCVDEKGGFIPGSLTARSLQIPQCPTTCEKSRTSGLLSSWKQARSQENPSPKDLFVPACLETGEYARLQASGAGTWCVDPASGEELRPGSSSSAQCPSLCNVLKSGVLSRRVSPGYVPACRAEDGGFSPVQCDQAQGSCWCVMDSGEEVPGTRVTGGQPACESPRCPLPFNASEVVGGTILCETISGPTGSAMQQCQLLCRQGSWSVFPPGPLICSLESGRWESQLPQPRACQRPQLWQTIQTQGHFQLQLPPGKMCSADYADLLQTFQVFILDELTARGFCQIQVKTFGTLVSIPVCNNSSVQVGCLTRERLGVNVTWKSRLEDIPVASLPDLHDIERALVGKDLLGRFTDLIQSGSFQLHLDSKTFPAETIRFLQGDHFGTSPRTWFGCSEGFYQVLTSEASQDGLGCVKCPEGSYSQDEECIPCPVGFYQEQAGSLACVPCPVGRTTISAGAFSQTHCVTDCQRNEAGLQCDQNGQYRASQKDRGSGKAFCVDGEGRRLPWWETEAPLEDSQCLMMQKFEKVPESKVIFDANAPVAVRSKVPDSEFPVMQCLTDCTEDEACSFFTVSTTEPEISCDFYAWTSDNVACMTSDQKRDALGNSKATSFGSLRCQVKVRSHGQDSPAVYLKKGQGSTTTLQKRFEPTGFQNMLSGLYNPIVFSASGANLTDAHLFCLLACDRDLCCDGFVLTQVQGGAIICGLLSSPSVLLCNVKDWMDPSEAWANATCPGVTYDQESHQVILRLGDQEFIKSLTPLEGTQDTFTNFQQVYLWKDSDMGSRPESMGCRKDTVPRPASPTEAGLTTELFSPVDLNQVIVNGNQSLSSQKHWLFKHLFSAQQANLWCLSRCVQEHSFCQLAEITESASLYFTCTLYPEAQVCDDIMESNAQGCRLILPQMPKALFRKKVILEDKVKNFYTRLPFQKLMGISIRNKVPMSEKSISNGFFECERRCDADPCCTGFGFLNVSQLKGGEVTCLTLNSLGIQMCSEENGGAWRILDCGSPDIEVHTYPFGWYQKPIAQNNAPSFCPLVVLPSLTEKVSLDSWQSLALSSVVVDPSIRHFDVAHVSTAATSNFSAVRDLCLSECSQHEACLITTLQTQPGAVRCMFYADTQSCTHSLQGQNCRLLLREEATHIYRKPGISLLSYEASVPSVPISTHGRLLGRSQAIQVGTSWKQVDQFLGVPYAAPPLAERRFQAPEPLNWTGSWDASKPRASCWQPGTRTSTSPGVSEDCLYLNVFIPQNVAPNASVLVFFHNTMDREESEGWPAIDGSFLAAVGNLIVVTASYRVGVFGFLSSGSGEVSGNWGLLDQVAALTWVQTHIRGFGGDPRRVSLAADRGGADVASIHLLTARATNSQLFRRAVLMGGSALSPAAVISHERAQQQAIALAKEVSCPMSSSQEVVSCLRQKPANVLNDAQTKLLAVSGPFHYWGPVIDGHFLREPPARALKRSLWVEVDLLIGSSQDDGLINRAKAVKQFEESRGRTSSKTAFYQALQNSLGGEDSDARVEAAATWYYSLEHSTDDYASFSRALENATRDYFIICPIIDMASAWAKRARGNVFMYHAPENYGHGSLELLADVQFALGLPFYPAYEGQFSLEEKSLSLKIMQYFSHFIRSGNPNYPYEFSRKVPTFATPWPDFVPRAGGENYKEFSELLPNRQGLKKADCSFWSKYISSLKTSADGAKGGQSAESEEEELTAGSGLREDLLSLQEPGSKTYSK

SEQ ID NO: 2 - protein, 9 aa, Homo sapiens
NLFGGKFLV

SEQ ID NO: 3 - protein, 6 aa, Mus musculus
DPNSYY

SEQ ID NO: 4 - protein, 7 aa, Mus musculus
VFSSTEI

SEQ ID NO: 5 - protein, 11 aa, Mus musculus
AVSSSGSWQLI

SEQ ID NO: 6 - protein, 5 aa, Mus musculus
KGHPV

SEQ ID NO: 7 - protein, 6 aa, Mus musculus
FQNQEV

SEQ ID NO: 8 - protein, 11 aa, Mus musculus
ASLGGSQDTQY

SEQ ID NO: 9 - protein, 123 aa, Mus musculus
MKTVTGPLFLCFWLQLNCVSRGEQVEQRPPHLSVREGDSAVIICTYTDPNSYYFFWYKQEPGAGLQLLMKVFSSTEINEGQGFTVLLNKKDKQLSLNLTAAHPGDSAVYFCAVSSSGSWQLIF

SEQ ID NO: 10 - protein, 123 aa, Mus musculus
MATRLLCYTVLCLLGARILNSKVIQTPRYLVKGQGQKAKMRCIPEKGHPVVFWYQQNKNNEFKFLINFQNQEVLQQIDMTEKRFSAECPSNSPCSLEIQSSEAGDSALYLCASLGGSQDTQYF

SEQ ID NO: 11 - protein, 270 aa, Mus musculus
MKTVTGPLFLCFWLQLNCVSRGEQVEQRPPHLSVREGDSAVIICTYTDPNSYYFFWYKQEPGAGLQLLMKVFSSTEINEGQGFTVLLNKKDKQLSLNLTAAHPGDSAVYFCAVSSSGSWQLIFGSGTQLTVMPDIQNPEPAVYQLKDPRSQDSTLCLFTDFDSQINVPKTMESGTFITDKTVLDMKAMDSKSNGAIAWSNQTSFTCQDIFKETNATYPSSDVPCDATLTEKSFETDMNLNFQNLSVMGLRILLLKVAGFNLLMTLRLWSS

SEQ ID NO: 12 - protein, 305 aa, Mus musculus
MATRLLCYTVLCLLGARILNSKVIQTPRYLVKGQGQKAKMRCIPEKGHPVVFWYQQNKNNEFKFLINFQNQEVLQQIDMTEKRFSAECPSNSPCSLEIQSSEAGDSALYLCASLGGSQDTQYFGPGTRLLVLEDLRNVTPPKVSLFEPSKAEIANKQKATLVCLARGFFPDHVELSWWVNGKEVHSGVSTDPQAYKESNYSYCLSSRLRVSATFWHNPRNHFRCQVQFHGLSEEDKWPEGSPKPVTQNISAEAWGRADCGITSASYHQGVLSATILYEILLGKATLYAVLVSGLVLMAMVKKKNS

SEQ ID NO: 13 - protein, 147 aa, Mus musculus
GSGTQLTVMPDIQNPEPAVYQLKDPRSQDSTLCLFTDFDSQINVPKTMESGTFITDKTVLDMKAMDSKSNGAIAWSNQTSFTCQDIFKETNATYPSSDVPCDATLTEKSFETDMNLNFQNLSVMGLRILLLKVAGFNLLMTLRLWSS

SEQ ID NO: 14 - protein, 182 aa, Mus musculus
GPGTRLLVLEDLRNVTPPKVSLFEPSKAEIANKQKATLVCLARGFFPDHVELSWWVNGKEVHSGVSTDPQAYKESNYSYCLSSRLRVSATFWHNPRNHFRCQVQFHGLSEEDKWPEGSPKPVTQNISAEAWGRADCGITSASYHQGVLSATILYEILLGKATLYAVLVSGLVLMAMVKKKNS

SEQ ID NO: 15 - DNA, 369 bp, Mus musculus
atgaagacagtgactggacctttgttcctgtgcttctggctgcagctgaactgtgtgagcagaggcgagcaggtggagcagcgccctcctcacctgagtgtccgggagggagacagtgccgttatcatctgcacctacacagaccctaacagttattacttcttctggtacaagcaagagccgggggcaggtcttcagttgcttatgaaggttttctcaagtacggaaataaacgaaggacaaggattcactgtcctactgaacaagaaagacaaacaactctctctgaacctcacagctgcccatcctggggactcagccgtgtacttctgcgcagtcagttcttctggcagctggcaactcatcttt

SEQ ID NO: 16 - DNA, 369 bp, Mus musculus
atggctacaaggctcctctgttacacagtactttgtctcctgggtgcaagaattttgaattcaaaagtcattcagactccaagatatctggtgaaagggcaaggacaaaaagcaaagatgaggtgtatccctgaaaagggacatccagttgtattctggtatcaacaaaataagaacaatgagtttaaatttttgattaactttcagaatcaagaagttcttcagcaaatagacatgactgaaaaacgattctctgctgagtgtccttcaaactcaccttgcagcctagaaattcagtcctctgaggcaggagactcagcactgtacctctgtgccagcctggggggaagccaagacacccagtacttt

SEQ ID NO: 17 - DNA, 813 bp, Mus musculus
atgaagacagtgactggacctttgttcctgtgcttctggctgcagctgaactgtgtgagcagaggcgagcaggtggagcagcgccctcctcacctgagtgtccgggagggagacagtgccgttatcatctgcacctacacagaccctaacagttattacttcttctggtacaagcaagagccgggggcaggtcttcagttgcttatgaaggttttctcaagtacggaaataaacgaaggacaaggattcactgtcctactgaacaagaaagacaaacaactctctctgaacctcacagctgcccatcctggggactcagccgtgtacttctgcgcagtcagttcttctggcagctggcaactcatctttggatctggaacccaactgacagttatgcctgacatccagaacccagaacctgctgtgtaccagttaaaagatcctcggtctcaggacagcaccctctgcctgttcaccgactttgactcccaaatcaatgtgccgaaaaccatggaatctggaacgttcatcactgacaaaactgtgctggacatgaaagctatggattccaagagcaatggggccattgcctggagcaaccagacaagcttcacctgccaagatatcttcaaagagaccaacgccacctaccccagttcagacgttccctgtgatgccacgttgactgagaaaagctttgaaacagatatgaacctaaactttcaaaacctgtcagttatgggactccgaatcctcctgctgaaagtagccggatttaacctgctcatgacgctgaggctgtggtccagttag

SEQ ID NO: 18 - DNA, 918 bp, Mus musculus
atggctacaaggctcctctgttacacagtactttgtctcctgggtgcaagaattttgaattcaaaagtcattcagactccaagatatctggtgaaagggcaaggacaaaaagcaaagatgaggtgtatccctgaaaagggacatccagttgtattctggtatcaacaaaataagaacaatgagtttaaatttttgattaactttcagaatcaagaagttcttcagcaaatagacatgactgaaaaacgattctctgctgagtgtccttcaaactcaccttgcagcctagaaattcagtcctctgaggcaggagactcagcactgtacctctgtgccagcctggggggaagccaagacacccagtactttgggccaggcactcggctcctcgtgttagaggatctgagaaatgtgactccacccaaggtctccttgtttgagccatcaaaagcagagattgcaaacaaacaaaaggctaccctcgtgtgcttggccaggggcttcttccctgaccacgtggagctgagctggtgggtgaatggcaaggaggtccacagtggggtcagcacggaccctcaggcctacaaggagagcaattatagctactgcctgagcagccgcctgagggtctctgctaccttctggcacaatcctcgaaaccacttccgctgccaagtgcagttccatgggctttcagaggaggacaagtggccagagggctcacccaaacctgtcacacagaacatcagtgcagaggcctggggccgagcagactgtggaatcacttcagcatcctatcatcagggggttctgtctgcaaccatcctctatgagatcctactggggaaggccaccctatatgctgtgctggtcagtggcctggtgctgatggccatggtcaagaaaaaaaattcctga

SEQ ID NO: 19 - DNA, 441 bp, Mus musculus
ggatctggaacccaactgacagttatgcctgacatccagaacccagaacctgctgtgtaccagttaaaagatcctcggtctcaggacagcaccctctgcctgttcaccgactttgactcccaaatcaatgtgccgaaaaccatggaatctggaacgttcatcactgacaaaactgtgctggacatgaaagctatggattccaagagcaatggggccattgcctggagcaaccagacaagcttcacctgccaagatatcttcaaagagaccaacgccacctaccccagttcagacgttccctgtgatgccacgttgactgagaaaagctttgaaacagatatgaacctaaactttcaaaacctgtcagttatgggactccgaatcctcctgctgaaagtagccggatttaacctgctcatgacgctgaggctgtggtccagt

SEQ ID NO: 20 - DNA, 549 bp, Mus musculus
gggccaggcactcggctcctcgtgttagaggatctgagaaatgtgactccacccaaggtctccttgtttgagccatcaaaagcagagattgcaaacaaacaaaaggctaccctcgtgtgcttggccaggggcttcttccctgaccacgtggagctgagctggtgggtgaatggcaaggaggtccacagtggggtcagcacggaccctcaggcctacaaggagagcaattatagctactgcctgagcagccgcctgagggtctctgctaccttctggcacaatcctcgaaaccacttccgctgccaagtgcagttccatgggctttcagaggaggacaagtggccagagggctcacccaaacctgtcacacagaacatcagtgcagaggcctggggccgagcagactgtggaatcacttcagcatcctatcatcagggggttctgtctgcaaccatcctctatgagatcctactggggaaggccaccctatatgctgtgctggtcagtggcctggtgctgatggccatggtcaagaaaaaaaattcctga

SEQ ID NO: 21 - DNA, 7394 bp, Artificial Sequence
  Synthetic
ccatgaagacagtgactggacctttgttcctgtgcttctggctgcagctgaactgtgtgagcagaggcgagcaggtggagcagcgccctcctcacctgagtgtccgggagggagacagtgccgttatcatctgcacctacacagaccctaacagttattacttcttctggtacaagcaagagccgggggcaggtcttcagttgcttatgaaggttttctcaagtacggaaataaacgaaggacaaggattcactgtcctactgaacaagaaagacaaacaactctctctgaacctcacagctgcccatcctggggactcagccgtgtacttctgcgcagtcagttcttctggcagctggcaactcatctttggatctggaacccaactgacagttatgcctgacatccagaacccagaacctgctgtgtaccagttaaaagatcctcggtctcaggacagcaccctctgcctgttcaccgactttgactcccaaatcaatgtgccgaaaaccatggaatctggaacgttcatcactgacaaaactgtgctggacatgaaagctatggattccaagagcaatggggccattgcctggagcaaccagacaagcttcacctgccaagatatcttcaaagagaccaacgccacctaccccagttcagacgttccctgtgatgccacgttgactgagaaaagctttgaaacagatatgaacctaaactttcaaaacctgtcagttatgggactccgaatcctcctgctgaaagtagccggatttaacctgctcatgacgctgaggctgtggtccagtcgggccaagcggtccggatccggagccaccaacttcagcctgctgaagcaggccggcgacgtggaggagaaccccggccccatggctacaaggctcctctgttacacagtactttgtctcctgggtgcaagaattttgaattcaaaagtcattcagactccaagatatctggtgaaagggcaaggacaaaaagcaaagatgaggtgtatccctgaaaagggacatccagttgtattctggtatcaacaaaataagaacaatgagtttaaatttttgattaactttcagaatcaagaagttcttcagcaaatagacatgactgaaaaacgattctctgctgagtgtccttcaaactcaccttgcagcctagaaattcagtcctctgaggcaggagactcagcactgtacctctgtgccagcctggggggaagccaagacacccagtactttgggccaggcactcggctcctcgtgttagaggatctgagaaatgtgactccacccaaggtctccttgtttgagccatcaaaagcagagattgcaaacaaacaaaaggctaccctcgtgtgcttggccaggggcttcttccctgaccacgtggagctgagctggtgggtgaatggcaaggaggtccacagtggggtcagcacggaccctcaggcctacaaggagagcaattatagctactgcctgagcagccgcctgagggtctctgctaccttctggcacaatcctcgaaaccacttccgctgccaagtgcagttccatgggctttcagaggaggacaagtggccagagggctcacccaaacctgtcacacagaacatcagtgcagaggcctggggccgagcagactgtggaatcacttcagcatcctatcatcagggggttctgtctgcaaccatcctctatgagatcctactggggaaggccaccctatatgctgtgctggtcagtggcctggtgctgatggccatggtcaagaaaaaaaattcctgaccgaattctgcagtcgacggtaccgcgggcccgggatcgatccgataaaataaaagattttatttagtctccagaaaaaggggggaatgaaagaccccacctgtaggtttggcaagctagcttaagtaacgccattttgcaaggcatggaaaatacataactgagaatagagaagttcagatcaaggttaggaacagagagacagcagaatatgggccaaacaggatatctgtggtaagcagttcctgccccggctcagggccaagaacagatggtccccagatgcggtcccgccctcagcagtttctagagaaccatcagatgtttccagggtgccccaaggacctgaaaatgaccctgtgccttatttgaactaaccaatcagttcgcttctcgcttctgttcgcgcgcttctgctccccgagctcaataaaagagcccacaacccctcactcggcgcgccagtcctccgatagactgcgtcgcccgggtacccgtgtatccaataaaccctcttgcagttgcatccgacttgtggtctcgctgttccttgggagggtctcctctgagtgattgactacccgtcagcgggggtctttcatgggtaacagtttcttgaagttggagaacaacattctgagggtaggagtcgaatattaagtaatcctgactcaattagccactgttttgaatccacatactccaatactcctgaaatccatcgatggagttcattatggacagcgcagaaagagctggggagaattgtgaaattgttatccgctcacaattccacacaacatacgagccggaagcataaagtgtaaagcctggggtgcctaatgagtgagctaactcacattaattgcgttgcgctcactgcccgctttccagtcgggaaacctgtcgtgccagctgcattaatgaatcggccaacgcgcggggagaggcggtttgcgtattgggcgctcttccgcttcctcgctcactgactcgctgcgctcggtcgttcggctgcggcgagcggtatcagctcactcaaaggcggtaatacggttatccacagaatcaggggataacgcaggaaagaacatgtgagcaaaaggccagcaaaaggccaggaaccgtaaaaaggccgcgttgctggcgtttttccataggctccgcccccctgacgagcatcacaaaaatcgacgctcaagtcagaggtggcgaaacccgacaggactataaagataccaggcgtttccccctggaagctccctcgtgcgctctcctgttccgaccctgccgcttaccggatacctgtccgcctttctcccttcgggaagcgtggcgctttctcatagctcacgctgtaggtatctcagttcggtgtaggtcgttcgctccaagctgggctgtgtgcacgaaccccccgttcagcccgaccgctgcgccttatccggtaactatcgtcttgagtccaacccggtaagacacgacttatcgccactggcagcagccactggtaacaggattagcagagcgaggtatgtaggcggtgctacagagttcttgaagtggtggcctaactacggctacactagaaggacagtatttggtatctgcgctctgctgaagccagttaccttcggaaaaagagttggtagctcttgatccggcaaacaaaccaccgctggtagcggtggtttttttgtttgcaagcagcagattacgcgcagaaaaaaaggatctcaagaagatcctttgatcttttctacggggtctgacgctcagtggaacgaaaactcacgttaagggattttggtcatgagattatcaaaaaggatcttcacctagatccttttaaattaaaaatgaagttttaaatcaatctaaagtatatatgagtaaacttggtctgacagttaccaatgcttaatcagtgaggcacctatctcagcgatctgtctatttcgttcatccatagttgcctgactccccgtcgtgtagataactacgatacgggagggcttaccatctggccccagtgctgcaatgataccgcgagacccacgctcaccggctccagatttatcagcaataaaccagccagccggaagggccgagcgcagaagtggtcctgcaactttatccgcctccatccagtctattaattgttgccgggaagctagagtaagtagttcgccagttaatagtttgcgcaacgttgttgccattgctacaggcatcgtggtgtcacgctcgtcgtttggtatggcttcattcagctccggttcccaacgatcaaggcgagttacatgatcccccatgttgtgcaaaaaagcggttagctccttcggtcctccgatcgttgtcagaagtaagttggccgcagtgttatcactcatggttatggcagcactgcataattctcttactgtcatgccatccgtaagatgcttttctgtgactggtgagtactcaaccaagtcattctgagaatagtgtatgcggcgaccgagttgctcttgcccggcgtcaatacgggataataccgcgccacatagcagaactttaaaagtgctcatcattggaaaacgttcttcggggcgaaaactctcaaggatcttaccgctgttgagatccagttcgatgtaacccactcgtgcacccaactgatcttcagcatcttttactttcaccagcgtttctgggtgagcaaaaacaggaaggcaaaatgccgcaaaaaagggaataagggcgacacggaaatgttgaatactcatactcttcctttttcaatattattgaagcatttatcagggttattgtctcatgagcggatacatatttgaatgtatttagaaaaataaacaaataggggttccgcgcacatttccccgaaaagtgccacctgacgtctaagaaaccattattatcatgacattaacctataaaaataggcgtatcacgaggccctttcgtctcgcgcgtttcggtgatgacggtgaaaacctctgacacatgcagctcccggagacggtcacagcttgtctgtaagcggatgccgggagcagacaagcccgtcagggcgcgtcagcgggtgttggcgggtgtcggggctggcttaactatgcggcatcagagcagattgtactgagagtgcaccatatgcggtgtgaaataccgcacagatgcgtaaggagaaaataccgcatcaggcgccattcgccattcaggctgcgcaactgttgggaagggcgatcggtgcgggcctcttcgctattacgccagctggcgaaagggggatgtgctgcaaggcgattaagttgggtaacgccagggttttcccagtcacgacgttgtaaaacgacggccagtgccacgctctcccttatgcgactcctgcattaggaagcagcccagtagtaggttgaggccgttgagcaccgccgccgcaaggaatggtgcatgcaaggagatggcgcccaacagtcccccggccacggggcctgccaccatacccacgccgaaacaagcgctcatgagcccgaagtggcgagcccgatcttccccatcggtgatgtcggcgatataggcgccagcaaccgcacctgtggcgccggtgatgccggccacgatgcgtccggcgtagaggcgatttaaagacaggatatcagtggtccaggctctagttttgactcaacaatatcaccagctgaagcctatagagtacgagccatagataaaataaaagattttatttagtctccagaaaaaggggggaatgaaagaccccacctgtaggtttggcaagctagcttaagtaacgccattttgcaaggcatggaaaatacataactgagaatagagaagttcagatcaaggttaggaacagagagacagcagaatatgggccaaacaggatatctgtggtaagcagttcctgccccggctcagggccaagaacagatggtccccagatgcggtcccgccctcagcagtttctagagaaccatcagatgtttccagggtgccccaaggacctgaaaatgaccctgtgccttatttgaactaaccaatcagttcgcttctcgcttctgttcgcgcgcttctgctccccgagctcaataaaagagcccacaacccctcactcggcgcgccagtcctccgatagactgcgtcgcccgggtacccgtattcccaataaagcctcttgctgtttgcatccgaatcgtggactcgctgatccttgggagggtctcctcagattgattgactgcccacctcgggggtctttcatttggaggttccaccgagatttggagacccctgcctagggaccaccgacccccccgccgggaggtaagctggccagcggtcgtttcgtgtctgtctctgtctttgtgcgtgtttgtgccggcatctaatgtttgcgcctgcgtctgtactagttagctaactagctctgtatctggcggacccgtggtggaactgacgagttcggaacacccggccgcaaccctgggagacgtcccagggacttcgggggccgtttttgtggcccgacctgagtccaaaaatcccgatcgttttggactctttggtgcaccccccttagaggagggatatgtggttctggtaggagacgagaacctaaaacagttcccgcctccgtctgaatttttgctttcggtttgggaccgaagccgcgccgcgcgtcttgtctgctgcagcatcgttctgtgttgtctctgtctgactgtgtttctgtatttgtctgagaatatgggcccgggctagcctgttaccactcccttaagtttgaccttaggtcactggaaagatgtcgagcggatcgctcacaaccagtcggtagatgtcaagaagagacgttgggttaccttctgctctgcagaatggccaacctttaacgtcggatggccgcgagacggcacctttaaccgagacctcatcacccaggttaagatcaaggtcttttcacctggcccgcatggacacccagaccaggtcccctacatcgtgacctgggaagccttggcttttgacccccctccctgggtcaagccctttgtacaccctaagcctccgcctcctcttcctccatccgccccgtctctcccccttgaacctcctcgttcgaccccgcctcgatcctccctttatccagccctcactccttctctaggcgcccccatatggccatatgagatcttatatggggcacccccgccccttgtaaacttccctgaccctgacatgacaagagttactaacagcccctctctccaagctcacttacaggctctctacttagtccagcacgaagtctggagacctctggcggcagcctaccaagaacaactggaccgaccggtggtacctcacccttaccgagtcggcgacacagtgtgggtccgccgacaccagactaagaacctagaacctcgctggaaaggaccttacacagtcctgctgaccacccccaccgccctcaaagtagacggcatcgcagcttggatacacgccgcccacgtgaaggctgccgaccccgggggtggaccatcctctagaccg

SEQ ID NO: 22 - DNA, 18 bp, Mus musculus
gaccctaacagttattac

SEQ ID NO: 23 - DNA, 21 bp, Mus musculus
gttttctcaagtacggaaata

SEQ ID NO: 24 - DNA, 33 bp, Mus musculus
gcagtcagttcttctggcagctggcaactcatc

SEQ ID NO: 25 - DNA, 15 bp, Mus musculus
aagggacatccagtt

SEQ ID NO: 26 - DNA, 18 bp, Mus musculus
tttcagaatcaagaagtt

SEQ ID NO: 27 - DNA, 33 bp, Mus musculus
gccagcctggggggaagccaagacacccagtac

SEQ ID NO: 28 - protein, 27 aa, Artificial Sequence
  Synthetic
RAKRSGSGATNFSLLKQAGDVEENPGP

SEQ ID NO: 29 - protein, 9 aa, Homo sapiens
TLLASICWV

SEQ ID NO: 30 - protein, 9 aa, Homo sapiens
ELPEFLLFL

SEQ ID NO: 31 - protein, 9 aa, Homo sapiens
ALVLEIFTL

SEQ ID NO: 32 - protein, 9 aa, Homo sapiens
ILQRRFLAV

SEQ ID NO: 33 - protein, 9 aa, Homo sapiens
ALLRSGPYM

SEQ ID NO: 34 - protein, 8 aa, Homo sapiens
LVEIFTLL

SEQ ID NO: 35 - protein, 9 aa, Homo sapiens
VQQVQCWCV

SEQ ID NO: 36 - DNA, 20 bp, Artificial Sequence
  Synthetic
ggctactttcagcaggagga

SEQ ID NO: 37 - DNA, 20 bp, Artificial Sequence
  Synthetic
aggcctctgcactgatgttc

SEQ ID NO: 38 - DNA, 41 bp, Artificial Sequence
  Synthetic
ccatcctctagaccgccatgaagacagtgactggacctttg

SEQ ID NO: 39 - DNA, 50 bp, Artificial Sequence
  Synthetic
tggtggctccggatccggaccgcttggcccgactggaccacagcctcagc

SEQ ID NO: 40 - DNA, 51 bp, Artificial Sequence
  Synthetic
gtaccgtcgactgcagaattcggtcaggaattttttttcttgaccatggcc

SEQ ID NO: 41 - DNA, 51 bp, Artificial Sequence
  Synthetic
gggccaagcggtccggatccggagccaccaacttcagcctgctgaagcagg

SEQ ID NO: 42 - DNA, 52 bp, Artificial Sequence
  Synthetic
accaacttcagcctgctgaagcaggccggcgacgtggaggagaaccccggcc

SEQ ID NO: 43 - DNA, 44 bp, Artificial Sequence
  Synthetic
tggaggagaaccccggccccatggctacaaggctcctctgttac

SEQ ID NO: 44 - protein, 6 aa, Homo sapiens
NSASQS

SEQ ID NO: 45 - protein, 6 aa, Homo sapiens
VYSSGN

SEQ ID NO: 46 - protein, 11 aa, Homo sapiens
VVHSSNTGKLI

SEQ ID NO: 47 - protein, 5 aa, Homo sapiens
MNHEY

SEQ ID NO: 48 - protein, 6 aa, Homo sapiens
SVGAGI

SEQ ID NO: 49 - protein, 18 aa, Homo sapiens
ASSYSLTSGGALVSYEQY

SEQ ID NO: 50 - protein, 121 aa, Homo sapiens
MISLRVLLVILWLQLSWVWSQRKEVEQDPGPFNVPEGATVAFNCTYSNSASQSFFWYRQDCRKEPKLLMSVYSSGNEDGRFTAQLNRASQYISLLIRDSKLSDSATYLCVVHSSNTGKLIF

SEQ ID NO: 51 - protein, 129 aa, Homo sapiens
MSIGLLCCAALSLLWAGPVNAGVTQTPKFQVLKTGQSMTLQCAQDMNHEYMSWYRQDPGMGLRLIHYSVGAGITDQGEVPNGYNVSRSTTEDFPLRLLSAAPSQTSVYFCASSYSLTSGGALVSYEQYF

SEQ ID NO: 52 - protein, 159 aa, Homo sapiens
GQGTTLQVKPDIQNPDPAVYQLRDSKSSDKSVCLFTDFDSQTNVSQSKDSDVYITDKTVLDMRSMDFKSNSAVAWSNKSDFACANAFNNSIIPEDTFFPSPESSCDVKLVEKSFETDTNLNFQNLSVIGFRILLLKVAGFNLLMTLRLWSSRAKRSGSG

SEQ ID NO: 53 - protein, 188 aa, Homo sapiens
GPGTRLTVTEDLKNVFPPEVAVFEPSEAEISHTQKATLVCLATGFYPDHVELSWWVNGKEVHSGVSTDPQPLKEQPALNDSRYCLSSRLRVSATFWQNPRNHFRCQVQFYGLSENDEWTQDRAKPVTQIVSAEAWGRADCGFTSESYQQGVLSATILYEILLGKATLYAVLVSALVLMAMVKRKDSRG

SEQ ID NO: 54 - protein, 280 aa, Homo sapiens
MISLRVLLVILWLQLSWVWSQRKEVEQDPGPFNVPEGATVAFNCTYSNSASQSFFWYRQDCRKEPKLLMSVYSSGNEDGRFTAQLNRASQYISLLIRDSKLSDSATYLCVVHSSNTGKLIFGQGTTLQVKPDIQNPDPAVYQLRDSKSSDKSVCLFTDFDSQTNVSQSKDSDVYITDKTVLDMRSMDFKSNSAVAWSNKSDFACANAFNNSIIPEDTFFPSPESSCDVKLVEKSFETDTNLNFQNLSVIGFRILLLKVAGFNLLMTLRLWSSRAKRSGSG

SEQ ID NO: 55 - protein, 317 aa, Homo sapiens
MSIGLLCCAALSLLWAGPVNAGVTQTPKFQVLKTGQSMTLQCAQDMNHEYMSWYRQDPGMGLRLIHYSVGAGITDQGEVPNGYNVSRSTTEDFPLRLLSAAPSQTSVYFCASSYSLTSGGALVSYEQYFGPGTRLTVTEDLKNVFPPEVAVFEPSEAEISHTQKATLVCLATGFYPDHVELSWWVNGKEVHSGVSTDPQPLKEQPALNDSRYCLSSRLRVSATFWQNPRNHFRCQVQFYGLSENDEWTQDRAKPVTQIVSAEAWGRADCGFTSESYQQGVLSATILYEILLGKATLYAVLVSALVLMAMVKRKDSRG

SEQ ID NO: 56 - DNA, 843 bp, Homo sapiens
atgatatccttgagagttttactggtgatcctgtggcttcagttaagctgggtttggagccaacggaaggaggtggagcaggatcctggacccttcaatgttccagagggagccactgtcgctttcaactgtacttacagcaacagtgcttctcagtctttcttctggtacagacaggattgcaggaaagaacctaagttgctgatgtccgtatactccagtggtaatgaagatggaaggtttacagcacagctcaatagagccagccagtatatttccctgctcatcagagactccaagctcagtgattcagccacctacctctgtgtggtccactctagcaacacaggcaaactaatctttgggcaagggacaactttacaagtaaaaccagatatccagaaccctgaccctgccgtgtaccagctgagagactctaaatccagtgacaagtctgtctgcctattcaccgattttgattctcaaacaaatgtgtcacaaagtaaggattctgatgtgtatatcacagacaaaactgtgctagacatgaggtctatggacttcaagagcaacagtgctgtggcctggagcaacaaatctgactttgcatgtgcaaacgccttcaacaacagcattattccagaagacaccttcttccccagcccagaaagttcctgtgatgtcaagctggtcgagaaaagctttgaaacagatacgaacctaaactttcaaaacctgtcagtgattgggttccgaatcctcctcctgaaagtggccgggtttaatctgctcatgacgctgcggctgtggtccagccgggccaagcggtccggatccggatga

SEQ ID NO: 57 - DNA, 954 bp, Homo sapiens
atgagcatcggcctcctgtgctgtgcagccttgtctctcctgtgggcaggtccagtgaatgctggtgtcactcagaccccaaaattccaggtcctgaagacaggacagagcatgacactgcagtgtgcccaggatatgaaccatgaatacatgtcctggtatcgacaagacccaggcatggggctgaggctgattcattactcagttggtgctggtatcactgaccaaggagaagtccccaatggctacaatgtctccagatcaaccacagaggatttcccgctcaggctgctgtcggctgctccctcccagacatctgtgtacttctgtgccagcagttactctttgactagcgggggggccttagtctcctacgagcagtacttcgggccgggcaccaggctcacggtcacagaggacctgaaaaacgtgttcccacccgaggtcgctgtgtttgagccatcagaagcagagatctcccacacccaaaaggccacactggtatgcctggccacaggcttctaccccgaccacgtggagctgagctggtgggtgaatgggaaggaggtgcacagtggggtcagcacagacccgcagcccctcaaggagcagcccgccctcaatgactccagatactgcctgagcagccgcctgagggtctcggccaccttctggcagaacccccgcaaccacttccgctgtcaagtccagttctacgggctctcggagaatgacgagtggacccaggatagggccaaacccgtcacccagatcgtcagcgccgaggcctggggtagagcagactgtggcttcacctccgagtcttaccagcaaggggtcctgtctgccaccatcctctatgagatcttgctagggaaggccaccttgtatgccgtgctggtcagtgccctcgtgctgatggctatggtcaagagaaaggattccagaggctag

SEQ ID NO: 58 - protein, 9 aa, Homo sapiens
LVLEIFTLL